European Patent Application EP 4 814 122 A1, published September 30, 2026. Title: MODIFIED TOMATO PLANTS. Applicant: Johann Wolfgang Goethe-Universität Frankfurt am Main. Application EP. The sequence listing filed with the application follows.

SEQUENCE LISTING (12 sequences)

SEQ ID NO: 1 - protein, 338 aa, Solanum lycopersicum
MTPQPIDRNKGETTAGETPRSVPTPFLTKTYQLIEDQSIDDVISWNEDGSTFIVWNPTEFARDLLPKYFKHNNFSSFVRQLNTYGFRKVVPDRWEFANDSFRRGERSQLVDIQRRKVATPIATPSAAATAVAIVASPPQPPPPPPSPSPPPPPPAQPPVAVSTSDSCEEQVLSSNSSAGSTAELLGENERLRLENLQLSKELNQMKKLCGNIYGMMSTYAHPSSSGNQSAESSSPSLKPLDLLGTERSVGESQVKAVEDRESHEVPEEAQARLFGFSIGMKRVREGEQAMMEHCHDLRLRQPGTTDVKVEPSDQESNGESEERSWLLHCGGRNQRTCN

SEQ ID NO: 2 - protein, 338 aa, synthetic construct; identical to SEQ ID NO: 1

SEQ ID NO: 3 - DNA, 1020 bp, Solanum lycopersicum
  source 1..1020: mol_type = other DNA
atgactccacagccaatagaccggaacaaaggagagacgacagccggtgaaacgccgaggtctgtgccgacaccgtttttaacaaagacctaccagctcatcgaggatcaatctattgacgatgtgatctcttggaatgaagacggatctacttttatagtgtggaatccaacggagttcgctagggatttgcttcctaaatattttaaacataataatttttctagcttcgttaggcagctcaacacctatggatttcggaaagtagtacctgatcgatgggaattcgcaaacgacagcttccggagaggtgagagaagtcagttagttgatatccagcgtcgaaaggttgccacgccgattgctactccttccgcagctgcaacagcggtggcgattgtggcttctccgcctcagcctccacctccacctccgtctccgtctccgcctccgcctccgcctgctcaaccaccggtggctgtatctacctctgattcctgtgaagagcaagttctatcgtcgaactcatctgcaggtagcacagcggagcttttaggagaaaacgaacggttaagattggagaatttacagctcagcaaagagttgaaccaaatgaagaagctctgcggcaatatatatggtatgatgtcgacttacgcacatccttcgagcagcggtaatcaatcggcggagagtagttcgccttcgttgaagccactggatctgttagggacggaacggtccgtaggtgaatctcaggtgaaggcggtagaggaccgggagagccatgaggtaccggaggaagcgcaggcgagattattcggtttctcgataggcatgaagcgtgttagggaaggggaacaagcaatgatggagcattgtcatgatttacggctgcggcaacctggaacaacggatgttaaagtagaaccgtctgatcaggaaagtaacggtgaaagtgaagagagatcgtggctgctacattgcggtggaagaaatcaaaggacttgtaattgatag

SEQ ID NO: 4 - DNA, 1131 bp, synthetic construct
  source 1..1131: mol_type = other DNA
atggtcttttacccatacgatgttcctgactatgcgggctatccctatgacgtcccggactatgcaggatcctatccatatgacgttccagattacgctgctcaggtaccgtcgagtactccacagccaatagaccggaacaaaggagagacgacagccggtgaaacgccgaggtctgtgccgacaccgtttttaacaaagacctaccagctcatcgaggatcaatctattgacgatgtgatctcttggaatgaagacggatctacttttatagtgtggaatccaacggagttcgctagggatttgcttcctaaatattttaaacataataatttttctagcttcgttaggcagctcaacacctatggatttcggaaagtagtacctgatcgatgggaattcgcaaacgacagcttccggagaggtgagagaagtcagttagttgatatccagcgtcgaaaggttgccacgccgattgctactccttccgcagctgcaacagcggtggcgattgtggcttctccgcctcagcctccacctccacctccgtctccgtctccgcctccgcctccgcctgctcaaccaccggtggctgtatctacctctgattcctgtgaagagcaagttctatcgtcgaactcatctgcaggtagcacagcggagcttttaggagaaaacgaacggttaagattggagaatttacagctcagcaaagagttgaaccaaatgaagaagctctgcggcaatatatatggtatgatgtcgacttacgcacatccttcgagcagcggtaatcaatcggcggagagtagttcgccttcgttgaagccactggatctgttagggacggaacggtccgtaggtgaatctcaggtgaaggcggtagaggaccgggagagccatgaggtaccggaggaagcgcaggcgagattattcggtttctcgataggcatgaagcgtgttagggaaggggaacaagcaatgatggagcattgtcatgatttacggctgcggcaacctggaacaacggatgttaaagtagaaccgtctgatcaggaaagtaacggtgaaagtgaagagagatcgtggctgctacattgcggtggaagaaatcaaaggacttgtaattga

SEQ ID NO: 5 - DNA, 58 bp, Solanum lycopersicum
  source 1..58: mol_type = other DNA
atgactccacagccaatagaccggaacaaaggagagacgacagccggtgaaacgccga

SEQ ID NO: 6 - DNA, 21 bp, synthetic construct
  source 1..21: mol_type = other DNA
atgactccacagccaatgagg

SEQ ID NO: 7 - DNA, 32 bp, synthetic construct
  source 1..32: mol_type = other DNA
taggtctctggagtaggctttacactttatgc

SEQ ID NO: 8 - DNA, 33 bp, synthetic construct
  source 1..33: mol_type = other DNA
tacggtctctagcgtacggtcacagcttgtctg

SEQ ID NO: 9 - DNA, 24 bp, synthetic construct
  source 1..24: mol_type = other DNA
ggaaagtagtacctgatcgatggg

SEQ ID NO: 10 - DNA, 22 bp, synthetic construct
  source 1..22: mol_type = other DNA
cagaggtagatacagccaccgg

SEQ ID NO: 11 - DNA, 20 bp, synthetic construct
  source 1..20: mol_type = other DNA
cgacagccggtgaaacgccg

SEQ ID NO: 12 - DNA, 20 bp, synthetic construct
  source 1..20: mol_type = other DNA
tgactccacagccaatagac